European Patent Specification EP 3 421 611 B1, published November 29, 2023. Title: Kit for diagnosis of leukemia and diagnostic method targeting prohibitin gene. Applicant: Industry Foundation of Chonnam National University Industry-Academic Cooperation Foundation of Dongshin University. The sequence listing filed with the application follows.

SEQUENCE LISTING (4 sequences)

SEQ ID NO: 1 - DNA, 19 bp, Artificial Sequence
  Prohibitin-1 FORWARD PRIMER
ggaggcgtggtgaactctg

SEQ ID NO: 2 - DNA, 20 bp, Artificial Sequence
  Prohibitin-1 BACKWARD PRIMER
ctggcacattacgtggtcga

SEQ ID NO: 3 - DNA, 20 bp, Artificial Sequence
  Prohibitin-2 FORWARD PRIMER
cttggttccagtaccccatt

SEQ ID NO: 4 - DNA, 19 bp, Artificial Sequence
  Prohibitin-2 BACKWARD PRIMER
cgagacaacactcgcaggg